European Patent Application EP 4 155 395 A1, published March 29, 2023. Title: Novel polypeptide and a method of producing L-leucine using the same. Applicant: CJ CheilJedang Corporation. The sequence listing filed with the application follows.

SEQUENCE LISTING (16 sequences)

SEQ ID NO: 1 - protein, 616 aa, Artificial Sequence
  LeuA AA (616 aa)
MSPNDAFISAPAKIETPVGPRNEGQPAWNKQRGSSMPVNRYMPFEVEVEDISLPDRTWPDKKITVAPQWCAVDLRDGNQALIDPMSPERKRRMFELLVQMGFKEIEVGFPSASQTDFDFVREIIEKGMIPDDVTIQVLVQAREHLIRRTFEACEGAKNVIVHFYNSTSILQRNVVFRMDKVQVKKLATDAAELIKTIAQDYPDTNWRWQYSPESFTGTEVEYAKEVVDAVVEVMDPTPENPMIINLPSTVEMITPNVYADSIEWMHRNLNRRDSIILSLHPHNDRGTGVGAAELGYMAGADRIEGCLFGNGERTGNVCLVTLALNMLTQGVDPQLDFTDIRQIRSTVEYCNQLRVPERHPYGGDLVFTAFSGSHQDAVNKGLDAMAAKVQPGASSTEVSWEQLRDTEWEVPYLPIDPKDVGRDYEAVIRVNSQSGKGGVAYIMKTDHGLQIPRSMQVEFSTVVQNVTDAEGGEVNSKAMWDIFATEYLERTAPVEQIALRVENAQTENEDASITAELIHNGKDVTVDGRGNGPLAAYANALEKLGIDVEIQEYNQHARTSGDDAEAAAYVLAEVNGRKVWGVGIAGSITYASLKAVTSAVNRALDVNHEAVLAGGV

SEQ ID NO: 2 - DNA, 1851 bp, Artificial Sequence
  leuA NT
atgtctcctaacgatgcattcatctccgcacctgccaagatcgaaaccccagttgggcctcgcaacgaaggccagccagcatggaataagcagcgtggctcctcaatgccagttaaccgctacatgcctttcgaggttgaggtagaagatatttctctgccggaccgcacttggccagataaaaaaatcaccgttgcacctcagtggtgtgctgttgacctgcgtgacggcaaccaggctctgattgatccgatgtctcctgagcgtaagcgccgcatgtttgagctgctggttcagatgggcttcaaagaaatcgaggtcggtttcccttcagcttcccagactgattttgatttcgttcgtgagatcatcgaaaagggcatgatccctgacgatgtcaccattcaggttctggttcaggctcgtgagcacctgattcgccgtacttttgaagcttgcgaaggcgcaaaaaacgttatcgtgcacttctacaactccacctccatcctgcagcgcaacgtggtgttccgcatggacaaggtgcaggtgaagaagctggctaccgatgccgctgaactaatcaagaccatcgctcaggattacccagacaccaactggcgctggcagtactcccctgagtccttcaccggcactgaggttgagtacgccaaggaagttgtggacgcagttgttgaggtcatggatccaactcctgagaacccaatgatcatcaacctgccttccaccgttgagatgatcacccctaacgtttacgcagactccattgaatggatgcaccgcaatctaaaccgtcgtgattccattatcctgtccctgcacccgcacaatgaccgtggcaccggcgttggcgcagctgagctgggctacatggctggcgctgaccgcatcgaaggctgcctgttcggcaacggcgagcgcaccggcaacgtctgcctggtcaccctggcactgaacatgctgacccagggcgttgaccctcagctggacttcaccgatatacgccagatccgcagcaccgttgaatactgcaaccagctgcgcgttcctgagcgccacccatacggcggtgacctggtcttcaccgctttctccggttcccaccaggacgctgtgaacaagggtctggacgccatggctgccaaggttcagccaggtgctagctccactgaagtttcttgggagcagctgcgcgacaccgaatgggaggttccttacctgcctatcgatccaaaggatgtcggtcgcgactacgaggctgttatccgcgtgaactcccagtccggcaagggcggcgttgcttacatcatgaagaccgatcacggtctgcagatccctcgctccatgcaggttgagttctccaccgttgtccagaacgtcaccgacgctgagggcggcgaggtcaactccaaggcaatgtgggatatcttcgccaccgagtacctggagcgcaccgcaccagttgagcagatcgcgctgcgcgtcgagaacgctcagaccgaaaacgaggatgcatccatcaccgccgagctcatccacaacggcaaggacgtcaccgtcgatggccgcggcaacggcccactggccgcttacgccaacgcgctggagaagctgggcatcgacgttgagatccaggaatacaaccagcacgcccgcacctcgggcgacgatgcagaagcagccgcctacgtgctggctgaggtcaacggccgcaaggtctggggcgtcggcatcgctggctccatcacctacgcttcgctgaaggcagtgacctccgccgtaaaccgcgcgctggacgtcaaccacgaggcagtcctggctggcggcgtttaa

SEQ ID NO: 3 - protein, 616 aa, Artificial Sequence
  LeuA P247C AA (616 aa)
MSPNDAFISAPAKIETPVGPRNEGQPAWNKQRGSSMPVNRYMPFEVEVEDISLPDRTWPDKKITVAPQWCAVDLRDGNQALIDPMSPERKRRMFELLVQMGFKEIEVGFPSASQTDFDFVREIIEKGMIPDDVTIQVLVQAREHLIRRTFEACEGAKNVIVHFYNSTSILQRNVVFRMDKVQVKKLATDAAELIKTIAQDYPDTNWRWQYSPESFTGTEVEYAKEVVDAVVEVMDPTPENPMIINLCSTVEMITPNVYADSIEWMHRNLNRRDSIILSLHPHNDRGTGVGAAELGYMAGADRIEGCLFGNGERTGNVCLVTLALNMLTQGVDPQLDFTDIRQIRSTVEYCNQLRVPERHPYGGDLVFTAFSGSHQDAVNKGLDAMAAKVQPGASSTEVSWEQLRDTEWEVPYLPIDPKDVGRDYEAVIRVNSQSGKGGVAYIMKTDHGLQIPRSMQVEFSTVVQNVTDAEGGEVNSKAMWDIFATEYLERTAPVEQIALRVENAQTENEDASITAELIHNGKDVTVDGRGNGPLAAYANALEKLGIDVEIQEYNQHARTSGDDAEAAAYVLAEVNGRKVWGVGIAGSITYASLKAVTSAVNRALDVNHEAVLAGGV

SEQ ID NO: 4 - DNA, 1851 bp, Artificial Sequence
  LeuA P247C NT
atgtctcctaacgatgcattcatctccgcacctgccaagatcgaaaccccagttgggcctcgcaacgaaggccagccagcatggaataagcagcgtggctcctcaatgccagttaaccgctacatgcctttcgaggttgaggtagaagatatttctctgccggaccgcacttggccagataaaaaaatcaccgttgcacctcagtggtgtgctgttgacctgcgtgacggcaaccaggctctgattgatccgatgtctcctgagcgtaagcgccgcatgtttgagctgctggttcagatgggcttcaaagaaatcgaggtcggtttcccttcagcttcccagactgattttgatttcgttcgtgagatcatcgaaaagggcatgatccctgacgatgtcaccattcaggttctggttcaggctcgtgagcacctgattcgccgtacttttgaagcttgcgaaggcgcaaaaaacgttatcgtgcacttctacaactccacctccatcctgcagcgcaacgtggtgttccgcatggacaaggtgcaggtgaagaagctggctaccgatgccgctgaactaatcaagaccatcgctcaggattacccagacaccaactggcgctggcagtactcccctgagtccttcaccggcactgaggttgagtacgccaaggaagttgtggacgcagttgttgaggtcatggatccaactcctgagaacccaatgatcatcaacctgtgttccaccgttgagatgatcacccctaacgtttacgcagactccattgaatggatgcaccgcaatctaaaccgtcgtgattccattatcctgtccctgcacccgcacaatgaccgtggcaccggcgttggcgcagctgagctgggctacatggctggcgctgaccgcatcgaaggctgcctgttcggcaacggcgagcgcaccggcaacgtctgcctggtcaccctggcactgaacatgctgacccagggcgttgaccctcagctggacttcaccgatatacgccagatccgcagcaccgttgaatactgcaaccagctgcgcgttcctgagcgccacccatacggcggtgacctggtcttcaccgctttctccggttcccaccaggacgctgtgaacaagggtctggacgccatggctgccaaggttcagccaggtgctagctccactgaagtttcttgggagcagctgcgcgacaccgaatgggaggttccttacctgcctatcgatccaaaggatgtcggtcgcgactacgaggctgttatccgcgtgaactcccagtccggcaagggcggcgttgcttacatcatgaagaccgatcacggtctgcagatccctcgctccatgcaggttgagttctccaccgttgtccagaacgtcaccgacgctgagggcggcgaggtcaactccaaggcaatgtgggatatcttcgccaccgagtacctggagcgcaccgcaccagttgagcagatcgcgctgcgcgtcgagaacgctcagaccgaaaacgaggatgcatccatcaccgccgagctcatccacaacggcaaggacgtcaccgtcgatggccgcggcaacggcccactggccgcttacgccaacgcgctggagaagctgggcatcgacgttgagatccaggaatacaaccagcacgcccgcacctcgggcgacgatgcagaagcagccgcctacgtgctggctgaggtcaacggccgcaaggtctggggcgtcggcatcgctggctccatcacctacgcttcgctgaaggcagtgacctccgccgtaaaccgcgcgctggacgtcaaccacgaggcagtcctggctggcggcgtttaa

SEQ ID NO: 5 - protein, 616 aa, Artificial Sequence
  LeuA P247C R558H G561D AA (616 aa)
MSPNDAFISAPAKIETPVGPRNEGQPAWNKQRGSSMPVNRYMPFEVEVEDISLPDRTWPDKKITVAPQWCAVDLRDGNQALIDPMSPERKRRMFELLVQMGFKEIEVGFPSASQTDFDFVREIIEKGMIPDDVTIQVLVQAREHLIRRTFEACEGAKNVIVHFYNSTSILQRNVVFRMDKVQVKKLATDAAELIKTIAQDYPDTNWRWQYSPESFTGTEVEYAKEVVDAVVEVMDPTPENPMIINLCSTVEMITPNVYADSIEWMHRNLNRRDSIILSLHPHNDRGTGVGAAELGYMAGADRIEGCLFGNGERTGNVCLVTLALNMLTQGVDPQLDFTDIRQIRSTVEYCNQLRVPERHPYGGDLVFTAFSGSHQDAVNKGLDAMAAKVQPGASSTEVSWEQLRDTEWEVPYLPIDPKDVGRDYEAVIRVNSQSGKGGVAYIMKTDHGLQIPRSMQVEFSTVVQNVTDAEGGEVNSKAMWDIFATEYLERTAPVEQIALRVENAQTENEDASITAELIHNGKDVTVDGRGNGPLAAYANALEKLGIDVEIQEYNQHAHTSDDDAEAAAYVLAEVNGRKVWGVGIAGSITYASLKAVTSAVNRALDVNHEAVLAGGV

SEQ ID NO: 6 - DNA, 1851 bp, Artificial Sequence
  LeuA P247C R558H G561D NT
atgtctcctaacgatgcattcatctccgcacctgccaagatcgaaaccccagttgggcctcgcaacgaaggccagccagcatggaataagcagcgtggctcctcaatgccagttaaccgctacatgcctttcgaggttgaggtagaagatatttctctgccggaccgcacttggccagataaaaaaatcaccgttgcacctcagtggtgtgctgttgacctgcgtgacggcaaccaggctctgattgatccgatgtctcctgagcgtaagcgccgcatgtttgagctgctggttcagatgggcttcaaagaaatcgaggtcggtttcccttcagcttcccagactgattttgatttcgttcgtgagatcatcgaaaagggcatgatccctgacgatgtcaccattcaggttctggttcaggctcgtgagcacctgattcgccgtacttttgaagcttgcgaaggcgcaaaaaacgttatcgtgcacttctacaactccacctccatcctgcagcgcaacgtggtgttccgcatggacaaggtgcaggtgaagaagctggctaccgatgccgctgaactaatcaagaccatcgctcaggattacccagacaccaactggcgctggcagtactcccctgagtccttcaccggcactgaggttgagtacgccaaggaagttgtggacgcagttgttgaggtcatggatccaactcctgagaacccaatgatcatcaacctgtgttccaccgttgagatgatcacccctaacgtttacgcagactccattgaatggatgcaccgcaatctaaaccgtcgtgattccattatcctgtccctgcacccgcacaatgaccgtggcaccggcgttggcgcagctgagctgggctacatggctggcgctgaccgcatcgaaggctgcctgttcggcaacggcgagcgcaccggcaacgtctgcctggtcaccctggcactgaacatgctgacccagggcgttgaccctcagctggacttcaccgatatacgccagatccgcagcaccgttgaatactgcaaccagctgcgcgttcctgagcgccacccatacggcggtgacctggtcttcaccgctttctccggttcccaccaggacgctgtgaacaagggtctggacgccatggctgccaaggttcagccaggtgctagctccactgaagtttcttgggagcagctgcgcgacaccgaatgggaggttccttacctgcctatcgatccaaaggatgtcggtcgcgactacgaggctgttatccgcgtgaactcccagtccggcaagggcggcgttgcttacatcatgaagaccgatcacggtctgcagatccctcgctccatgcaggttgagttctccaccgttgtccagaacgtcaccgacgctgagggcggcgaggtcaactccaaggcaatgtgggatatcttcgccaccgagtacctggagcgcaccgcaccagttgagcagatcgcgctgcgcgtcgagaacgctcagaccgaaaacgaggatgcatccatcaccgccgagctcatccacaacggcaaggacgtcaccgtcgatggccgcggcaacggcccactggccgcttacgccaacgcgctggagaagctgggcatcgacgttgagatccaggaatacaaccagcacgcccacacctcggatgacgatgcagaagcagccgcctacgtgctggctgaggtcaacggccgcaaggtctggggcgtcggcatcgctggctccatcacctacgcttcgctgaaggcagtgacctccgccgtaaaccgcgcgctggacgtcaaccacgaggcagtcctggctggcggcgtttaa

SEQ ID NO: 7 - DNA, 30 bp, Artificial Sequence
  pCR-leuA_F
ctaatctcgaggtcacccatgtctcctaac

SEQ ID NO: 8 - DNA, 27 bp, Artificial Sequence
  pCR-leuA_R
ggctggcggcgtttaaaaccggttgat

SEQ ID NO: 9 - DNA, 22 bp, Artificial Sequence
  leuA_sequencing_F
aacacgaccggcatcccgtcgc

SEQ ID NO: 10 - DNA, 23 bp, Artificial Sequence
  leuA_sequencing_R
aaatcatttgagaaaactcgagg

SEQ ID NO: 11 - DNA, 45 bp, Artificial Sequence
  leuA_P247C_Up_F
gtgaattcgagctcggtacccaaatcatttgagaaaactcgaggc

SEQ ID NO: 12 - DNA, 45 bp, Artificial Sequence
  leuA_P247C_Up_R
ggtgatcatctcaacggtggaacacaggttgatgatcattgggtt

SEQ ID NO: 13 - DNA, 45 bp, Artificial Sequence
  leuA_P247C_Down_F
aacccaatgatcatcaacctgtgttccaccgttgagatgatcacc

SEQ ID NO: 14 - DNA, 42 bp, Artificial Sequence
  leuA_P247C_Down_R
ggtcgactctagaggatccccaagaaggcaacatcggacagc

SEQ ID NO: 15 - DNA, 21 bp, Artificial Sequence
  leuA_sequencing_R
atccattcaatggagtctgcg

SEQ ID NO: 16 - protein, 581 aa, Artificial Sequence
  LeuA AA (581 aa)
MPVNRYMPFEVEVEDISLPDRTWPDKKITVAPQWCAVDLRDGNQALIDPMSPERKRRMFELLVQMGFKEIEVGFPSASQTDFDFVREIIEKGMIPDDVTIQVLVQAREHLIRRTFEACEGAKNVIVHFYNSTSILQRNVVFRMDKVQVKKLATDAAELIKTIAQDYPDTNWRWQYSPESFTGTEVEYAKEVVDAVVEVMDPTPENPMIINLPSTVEMITPNVYADSIEWMHRNLNRRDSIILSLHPHNDRGTGVGAAELGYMAGADRIEGCLFGNGERTGNVCLVTLALNMLTQGVDPQLDFTDIRQIRSTVEYCNQLRVPERHPYGGDLVFTAFSGSHQDAVNKGLDAMAAKVQPGASSTEVSWEQLRDTEWEVPYLPIDPKDVGRDYEAVIRVNSQSGKGGVAYIMKTDHGLQIPRSMQVEFSTVVQNVTDAEGGEVNSKAMWDIFATEYLERTAPVEQIALRVENAQTENEDASITAELIHNGKDVTVDGRGNGPLAAYANALEKLGIDVEIQEYNQHARTSGDDAEAAAYVLAEVNGRKVWGVGIAGSITYASLKAVTSAVNRALDVNHEAVLAGGV